European Patent Specification EP 3 417 934 B1, published December 27, 2023. Title: Encapsulation Vesicle and Production thereof. Applicant: Japan Science and Technology Agency. The sequence listing filed with the application follows.

SEQUENCE LISTING (4 sequences)

SEQ ID NO: 1 - RNA, 21 nt, Artificial
  the sense strand of a double-strand siRNA designed to target Fire fly luciferase gene
  misc_feature (20)..(20): n stands for deoxythymidine
  misc_feature (21)..(21): n stands for deoxythymidine
cuuacgcugaguacuucgann

SEQ ID NO: 2 - RNA, 21 nt, Artificial
  the antisense strand of a double-strand siRNA designed to target Firefly luciferase gene
  misc_feature (20)..(20): n stands for deoxythymidine
  misc_feature (21)..(21): n stands for deoxythymidine
ucgaaguacucagcguaagnn

SEQ ID NO: 3 - RNA, 21 nt, Artificial
  the sense strand of a scrumble siRNA
  misc_feature (20)..(20): n stands for deoxythymidine
  misc_feature (21)..(21): n stands for deoxythymidine
uucuccgaacgugucacgunn

SEQ ID NO: 4 - RNA, 21 nt, Artificial
  the antisense strand of a scrumble siRNA
  misc_feature (20)..(20): n stands for deoxythymidine
  misc_feature (21)..(21): n stands for deoxythymidine
acgugacacguucggagaann